European Patent Application EP 4 134 450 A1, published February 15, 2023. Title: Prediction of cancer-associated venous thromboembolism. Applicant: GENINCODE UK Limited. The sequence listing filed with the application follows.

SEQUENCE LISTING (18 sequences)

SEQ ID NO: 1 - DNA, 51 bp, Homo sapiens
  rs4524 risk allele
cttatgcttagcatgttcttgacttctgaattctccagcaccaagtgaaag

SEQ ID NO: 2 - DNA, 51 bp, Homo sapiens
  rs4524 non-risk allele
cttatgcttagcatgttcttgacttttgaattctccagcaccaagtgaaag

SEQ ID NO: 3 - DNA, 50 bp, Homo sapiens
  rs6025 risk allele
tgtaagagcagatccctggacaggcaaggaatacaggtattttgtccttg

SEQ ID NO: 4 - DNA, 50 bp, Homo sapiens
  rs6025 non-risk allele
tgtaagagcagatccctggacaggcgaggaatacaggtattttgtccttg

SEQ ID NO: 5 - DNA, 51 bp, Homo sapiens
  rs2232698 risk allele
ttcaaacttcggattcagcctgctgtgaaagatctccatgaggcacgatgg

SEQ ID NO: 6 - DNA, 51 bp, Homo sapiens
  rs2232698 non-risk allele
ttcaaacttcggattcagcctgctgcgaaagatctccatgaggcacgatgg

SEQ ID NO: 7 - DNA, 51 bp, Homo sapiens
  rs2227631 risk allele
ccccaagtcctagcgggcagctcgaagaagtgaaacttacacgttggtctc

SEQ ID NO: 8 - DNA, 51 bp, Homo sapiens
  rs2227631 non-risk allele
ccccaagtcctagcgggcagctcgaggaagtgaaacttacacgttggtctc

SEQ ID NO: 9 - DNA, 50 bp, Homo sapiens
  rs268 risk allele
tgcaacaatctgggctatgagatcagtaaagtcagagccaaaagaagcag

SEQ ID NO: 10 - DNA, 50 bp, Homo sapiens
  rs268 non-risk allele
tgcaacaatctgggctatgagatcaataaagtcagagccaaaagaagcag

SEQ ID NO: 11 - DNA, 51 bp, Homo sapiens
  rs169713 risk allele
tattattcgcactctacacagccagcgtggggattaatggcatgatgtgct

SEQ ID NO: 12 - DNA, 51 bp, Homo sapiens
  rs169713 non-risk allele
tattattcgcactctacacagccagtgtggggattaatggcatgatgtgct

SEQ ID NO: 13 - DNA, 51 bp, Homo sapiens
  rs11696364 risk allele
gctactaaaactaaacacagacttaactgatgaccaggtatttacccaaga

SEQ ID NO: 14 - DNA, 51 bp, Homo sapiens
  rs11696364 non-risk allele
gctactaaaactaaacacagacttacctgatgaccaggtatttacccaaga

SEQ ID NO: 15 - DNA, 51 bp, Homo sapiens
  rs5110 risk allele
gcacctgctcctgctgctgctcctgatgctgttcctgctgttgctccagct

SEQ ID NO: 16 - DNA, 51 bp, Homo sapiens
  rs5110 non-risk allele
gcacctgctcctgctgctgctcctgctgctgttcctgctgttgctccagct

SEQ ID NO: 17 - DNA, 51 bp, Homo sapiens
  rs6003 risk allele
tttgtaccctgaagcgcaaccataatgcatgttctcttgaattttatacaa

SEQ ID NO: 18 - DNA, 51 bp, Homo sapiens
  rs6003 non-risk allele
tttgtaccctgaagcgcaaccataacgcatgttctcttgaattttatacaa